European Patent Specification EP 3 448 876 B1, published March 6, 2024. Title: Streptavidin muteins and methods of using them. Applicant: IBA GmbH. The sequence listing filed with the application follows.

SEQUENCE LISTING (100 sequences)

SEQ ID NO: 1 - protein, 159 aa, artificial sequence
  mature wild-type streptavidin (residues 1 to 159)
DPSKDSKAQVSAAEAGITGTWYNQLGSTFIVTAGADGALTGTYESAVGNAESRYVLTGRYDSAPATDGSGTALGWTVAWKNNYRNAHSATTWSGQYVGGAEARINTQWLLTSGTTEANAWKSTLVGHDTFTKVKPSAASIDAAKKAGVNNGNPLDAVQQ

SEQ ID NO: 2 - protein, 126 aa, artificial sequence
  mature wild-type streptavidin (residues 14 to 139)
EAGITGTWYNQLGSTFIVTAGADGALTGTYESAVGNAESRYVLTGRYDSAPATDGSGTALGWTVAWKNNYRNAHSATTWSGQYVGGAEARINTQWLLTSGTTEANAWKSTLVGHDTFTKVKPSAAS

SEQ ID NO: 3 - protein, 8 aa, artificial sequence
  Step-tag II affinity tag
WSHPQFEK

SEQ ID NO: 4 - protein, 8 aa, artificial sequence
  Strep-tag affinity tag
WRHPQFGG

SEQ ID NO: 5 - protein, 28 aa, artificial sequence
  di-tag3 sequence
WSHPQFEKGGGSGGGSGGGSWSHPQFEK

SEQ ID NO: 6 - protein, 24 aa, artificial sequence
  di-tag2 sequence
WSHPQFEKGGGSGGGSWSHPQFEK

SEQ ID NO: 7 - protein, 28 aa, artificial sequence
  Twin-Strep-tag
WSHPQFEKGGGSGGGSGGSAWSHPQFEK

SEQ ID NO: 8 - protein, 8 aa, artificial sequence
  peptide sequence
  MISC_FEATURE (2)..(2): arbitrary amino acid
  MISC_FEATURE (7)..(8): position 7 and 8 G or position 7 E and position 8 R or K
WXHPQFXX

SEQ ID NO: 9 - protein, 8 aa, artificial sequence
  binding molecule
  MISC_FEATURE (1)..(1): position 1 is W, K or R
  MISC_FEATURE (2)..(2): any amino acid
  MISC_FEATURE (7)..(8): positions 7 and 8 both G or position 7 E and position 8 K or R
XXHPQFXX

SEQ ID NO: 10 - protein, 4 aa, artificial sequence
  amino acid position 44 to 47 of wild type streptavidin
VTAR

SEQ ID NO: 11 - protein, 4 aa, artificial sequence
  mutein of wildtype streptavidin at amino acid positions 44 to 47
IGAR

SEQ ID NO: 12 - protein, 126 aa, artificial sequence
  mutein "1"
EAGITGTWYNQLGSTFIVTAGADGALTGTYVTARGNAESRYVLTGRYDSAPATDGSGTALGWTVAWKNNYRNAHSATTWSGQYVGGAEARINTQWLLTSGTTEANAWKSTLVGHDTFTKVKPSAAS

SEQ ID NO: 13 - protein, 124 aa, artificial sequence
  mutein m302
EAGITGTWYNQLGSTFIVTAGADGALTGTYVTARGNAESRYVLTGRYDSAPATDGSGTALGWTVAWKNNYRNAHSATTWSGQYVGGAEARINTQWLLTSGTTEHWYSTLVGHDTFTKVKPSAAS

SEQ ID NO: 14 - protein, 124 aa, artificial sequence
  mutein m302C
EAGITGTWYNQLGSTFIVTAGADGALTGTYVTARGNAESRYVLTGRYDSAPATDGSGTALGWTVAWKNNYRNAHSATTWSGQYVGGAEARINTQWLLTSGTTEHWYSTLVGCDTFTKVKPSAAS

SEQ ID NO: 15 - protein, 126 aa, artificial sequence
  mutein m1-9
EAGITGTWYNQLGSTFIVTAGADGALTGTYVTARGNAESRYVLTGRYDSAPATDGSGTALGWTVAWKNNYRNAHSATTWSGQYVGGAEARINTQWLLTSGTTEENAGYSTLVGHDTFTKVKPSAAS

SEQ ID NO: 16 - protein, 126 aa, artificial sequence
  mutein m1-9C
EAGITGTWYNQLGSTFIVTAGADGALTGTYVTARGNAESRYVLTGRYDSAPATDGSGTALGWTVAWKNNYRNAHSATTWSGQYVGGAEARINTQWLLTSGTTEENAGYSTLVGCDTFTKVKPSAAS

SEQ ID NO: 17 - protein, 8 aa, artificial sequence
  sequence positions 114 to 121 of streptavidin
TTEANAWK

SEQ ID NO: 18 - protein, 14 aa, artificial sequence
  amino acid positions 114 to 121 of streptavidin replaced by this sequence according to Fletcher et al.
HPYFYAPELLFFAK

SEQ ID NO: 19 - protein, 16 aa, artificial sequence
  amino acid positions 114 to 121 of streptavidin replaced by this sequence according to Fletcher et al.
EGGKETLTPSELRDLV

SEQ ID NO: 20 - protein, 5 aa, artificial sequence
  wild type streptavidin (positions 117 to 121)
ANAWK

SEQ ID NO: 21 - protein, 5 aa, Artificial Sequence
  m36 fragment
YNAFM

SEQ ID NO: 22 - protein, 5 aa, Artificial Sequence
  m23 fragment
YNAYA

SEQ ID NO: 23 - protein, 5 aa, Artificial Sequence
  m41 fragment
  MISC_FEATURE (2)..(3): amino acid deletion
AXXWY

SEQ ID NO: 24 - protein, 5 aa, Artificial Sequence
  m4 fragment
DNAGF

SEQ ID NO: 25 - protein, 5 aa, Artificial Sequence
  m12 fragment
RNAGF

SEQ ID NO: 26 - protein, 5 aa, Artificial Sequence
  m22 fragment
QNAGF

SEQ ID NO: 27 - protein, 5 aa, Artificial Sequence
  m31 fragment
FNASW

SEQ ID NO: 28 - protein, 5 aa, Artificial Sequence
  m32 fragment
DNAVM

SEQ ID NO: 29 - protein, 5 aa, Artificial Sequence
  m35 fragment
  MISC_FEATURE (2)..(3): amino acid deletion
AXXWM

SEQ ID NO: 30 - protein, 5 aa, Artificial Sequence
  m38 fragment
ENAGF

SEQ ID NO: 31 - protein, 5 aa, Artificial Sequence
  m40 fragment
YNAYS

SEQ ID NO: 32 - protein, 5 aa, Artificial Sequence
  m 42 fragment
FNAYG

SEQ ID NO: 33 - protein, 5 aa, Artificial Sequence
  m45 fragment
YNAGF

SEQ ID NO: 34 - protein, 5 aa, Artificial Sequence
  m46 fragment
RNAYA

SEQ ID NO: 35 - protein, 5 aa, Artificial Sequence
  m47 fragment
WNAYG

SEQ ID NO: 36 - protein, 5 aa, Artificial Sequence
  m7 fragment
LNAGF

SEQ ID NO: 37 - protein, 5 aa, Artificial Sequence
  m10 fragment
HNAGY

SEQ ID NO: 38 - protein, 5 aa, Artificial Sequence
  m17 fragment
MNAGF

SEQ ID NO: 39 - protein, 5 aa, Artificial Sequence
  m21 fragment
RNAGY

SEQ ID NO: 40 - protein, 5 aa, Artificial Sequence
  m24 fragment
ENAGW

SEQ ID NO: 41 - protein, 5 aa, Artificial Sequence
  m27 fragment
HNAGF

SEQ ID NO: 42 - protein, 5 aa, Artificial Sequence
  m28 fragment
SNAGF

SEQ ID NO: 43 - protein, 5 aa, Artificial Sequence
  m30 fragment
TNAGF

SEQ ID NO: 44 - protein, 5 aa, Artificial Sequence
  m33 fragment
NNAGF

SEQ ID NO: 45 - protein, 5 aa, Artificial Sequence
  m1 frag,ent
ENAGM

SEQ ID NO: 46 - protein, 5 aa, Artificial Sequence
  m3 fragment
WNACC

SEQ ID NO: 47 - protein, 5 aa, Artificial Sequence
  m8 fragment
MNAFV

SEQ ID NO: 48 - protein, 5 aa, Artificial Sequence
  m15 fragment
ANADW

SEQ ID NO: 49 - protein, 5 aa, Artificial Sequence
  m6 fragment
SNAMM

SEQ ID NO: 50 - protein, 5 aa, Artificial Sequence
  m9 fragment
RNAVV

SEQ ID NO: 51 - protein, 5 aa, Artificial Sequence
  m20 fragment
SNASF

SEQ ID NO: 52 - protein, 5 aa, Artificial Sequence
  m34 fragment
  MISC_FEATURE (2)..(3): amino acid deletion
AXXWD

SEQ ID NO: 53 - protein, 5 aa, Artificial Sequence
  m14 fragment
RNARA

SEQ ID NO: 54 - protein, 5 aa, Artificial Sequence
  m18 fragment
SNAAF

SEQ ID NO: 55 - protein, 5 aa, Artificial Sequence
  m19 fragment
GNAMM

SEQ ID NO: 56 - protein, 5 aa, Artificial Sequence
  m8 fragment
ENAGF

SEQ ID NO: 57 - protein, 5 aa, Artificial Sequence
  m21 fragment
DNAGY

SEQ ID NO: 58 - protein, 5 aa, Artificial Sequence
  m9 fragment
ENAGY

SEQ ID NO: 59 - protein, 5 aa, Artificial Sequence
  m1 fragment
RNAMM

SEQ ID NO: 60 - protein, 5 aa, Artificial Sequence
  m2 fragment
RNAGF

SEQ ID NO: 61 - protein, 5 aa, Artificial Sequence
  m3 fragment
ANAPA

SEQ ID NO: 62 - protein, 5 aa, Artificial Sequence
  m5 fragment
ANAMV

SEQ ID NO: 63 - protein, 5 aa, Artificial Sequence
  m13 fragment
QNASA

SEQ ID NO: 64 - protein, 5 aa, Artificial Sequence
  m14 fragment
ANAGF

SEQ ID NO: 65 - protein, 5 aa, Artificial Sequence
  m24 fragemnt
QNAMV

SEQ ID NO: 66 - protein, 5 aa, Artificial Sequence
  m4 fragment
NNAGY

SEQ ID NO: 67 - protein, 5 aa, Artificial Sequence
  m6 fragment
ANAAV

SEQ ID NO: 68 - protein, 5 aa, Artificial Sequence
  m7 fragment
SNAMI

SEQ ID NO: 69 - protein, 5 aa, Artificial Sequence
  m10 fragment
HNAGY

SEQ ID NO: 70 - protein, 5 aa, Artificial Sequence
  m15 fragment
SNAMA

SEQ ID NO: 71 - protein, 5 aa, Artificial Sequence
  m23 fragment
QNAVA

SEQ ID NO: 72 - protein, 5 aa, Artificial Sequence
  m17 fragment
YNAYM

SEQ ID NO: 73 - protein, 5 aa, Artificial Sequence
  m12 fragment
LNAWG

SEQ ID NO: 74 - protein, 5 aa, Artificial Sequence
  m20 fragment
HNASM

SEQ ID NO: 75 - protein, 5 aa, Artificial Sequence
  m101 fragment
YNAFL

SEQ ID NO: 76 - protein, 5 aa, Artificial Sequence
  m106 fragment
FNAFL

SEQ ID NO: 77 - protein, 5 aa, Artificial Sequence
  m111 fragment
YNALW

SEQ ID NO: 78 - protein, 5 aa, Artificial Sequence
  m100 fragment
FNAYI

SEQ ID NO: 79 - protein, 5 aa, Artificial Sequence
  m110 fragment
YNAYL

SEQ ID NO: 80 - protein, 5 aa, Artificial Sequence
  m104 fragment
YNAYQ

SEQ ID NO: 81 - protein, 5 aa, Artificial Sequence
  m108 fragment
FNAIW

SEQ ID NO: 82 - protein, 5 aa, Artificial Sequence
  m207 fragment
  MISC_FEATURE (2)..(3): amino acid deletion
TXXWL

SEQ ID NO: 83 - protein, 5 aa, Artificial Sequence
  m212 fragment
  MISC_FEATURE (2)..(3): amino acid deletion
HXXWL

SEQ ID NO: 84 - protein, 5 aa, Artificial Sequence
  m202 fragment
  MISC_FEATURE (2)..(3): amino acid deletion
IXXWR

SEQ ID NO: 85 - protein, 5 aa, Artificial Sequence
  m204 fragment
  MISC_FEATURE (2)..(3): amino acid deletion
HXXWT

SEQ ID NO: 86 - protein, 5 aa, Artificial Sequence
  m206 fragment
  MISC_FEATURE (2)..(3): amino acid deletion
TXXWR

SEQ ID NO: 87 - protein, 5 aa, Artificial Sequence
  m208 fragment
  MISC_FEATURE (2)..(3): amino acid deletion
AXXWR

SEQ ID NO: 88 - protein, 5 aa, Artificial Sequence
  m203 fragment
  MISC_FEATURE (2)..(3): amino acid deletion
RXXWS

SEQ ID NO: 89 - protein, 5 aa, Artificial Sequence
  m209 fragment
  MISC_FEATURE (2)..(3): amino acid deletion
NXXWR

SEQ ID NO: 90 - protein, 5 aa, Artificial Sequence
  m200 fragment
  MISC_FEATURE (2)..(3): amino acid deletion
KXXWS

SEQ ID NO: 91 - protein, 5 aa, Artificial Sequence
  m201 fragment
  MISC_FEATURE (2)..(3): amino acid deletion
SXXVF

SEQ ID NO: 92 - protein, 5 aa, Artificial Sequence
  m211 fragment
  MISC_FEATURE (2)..(3): amino acid deletion
KXXWT

SEQ ID NO: 93 - protein, 5 aa, Artificial Sequence
  m300 fragment
  MISC_FEATURE (2)..(3): amino acid deletion
AXXWY

SEQ ID NO: 94 - protein, 5 aa, Artificial Sequence
  m301 fragment
  MISC_FEATURE (2)..(3): amino acid deletion
HXXWM

SEQ ID NO: 95 - protein, 5 aa, Artificial Sequence
  m302 fragment
  MISC_FEATURE (2)..(3): amino acid deletion
HXXWY

SEQ ID NO: 96 - protein, 5 aa, Artificial Sequence
  m303 fragment
  MISC_FEATURE (2)..(3): amino acid deletion
EXXWY

SEQ ID NO: 97 - protein, 5 aa, Artificial Sequence
  m304 fragment
  MISC_FEATURE (2)..(3): amino acid deletion
QXXWY

SEQ ID NO: 98 - protein, 5 aa, artificial sequence
  motif 1 (figure 2)
  MISC_FEATURE (1)..(1): position 1 is E,D, R, H, N, Q, T, S, L or M
  MISC_FEATURE (5)..(5): position 5 is F, Y or M
XNAGX

SEQ ID NO: 99 - protein, 5 aa, artificial sequence
  motif 2 (figure 2)
  MISC_FEATURE (1)..(1): position 1 is Y, F, R, W or Q
  MISC_FEATURE (4)..(4): position 4 is Y, F, L, I or M
  MISC_FEATURE (5)..(5): position 5 is L, I, M, Q, G, W, S, A or V
XNAXX

SEQ ID NO: 100 - protein, 5 aa, artificial sequence
  motif 3, consensus sequence 3
  MISC_FEATURE (1)..(1): any amino acid
  MISC_FEATURE (1)..(1): any amino acid, preferably H, E, Q, T, A or I
  MISC_FEATURE (2)..(3): amino acid deletion
  MISC_FEATURE (4)..(4): position 4 is W or V
  MISC_FEATURE (5)..(5): any amino acid, preferably Y, L, M or R
XXXXX